European Patent Application EP 4 570 266 A1, published June 18, 2025. Title: Antibody targeting extracellular cyclophilin A. Applicant: Eberhard Karls Universität Tübingen, Medizinische Fakultät. Application EP. The sequence listing filed with the application follows.

SEQUENCE LISTING (18 sequences)

SEQ ID NO: 1 - protein, 8 aa, synthetic construct
HFATVESY

SEQ ID NO: 2 - protein, 9 aa, synthetic construct
MQATHAPWT

SEQ ID NO: 3 - protein, 16 aa, synthetic construct
YITRSSDTVYADAVKG

SEQ ID NO: 4 - protein, 7 aa, synthetic construct
LVSNLGS

SEQ ID NO: 5 - protein, 5 aa, synthetic construct
RYGMH

SEQ ID NO: 6 - protein, 16 aa, synthetic construct
RSSQSLLDSDGNTYLY

SEQ ID NO: 7 - protein, 135 aa, synthetic construct
MYFSISLFFLVLILKSVQCEVQLVESGGGLVQPGKSLKLSCSASGFTFSRYGMHWIRQAPGKGLDWVAYITRSSDTVYADAVKGRFTISRDNAKSTLYLQLNSLKSEDTAIYYCASHFATVESYWGQGVMVTVSS

SEQ ID NO: 8 - protein, 131 aa, synthetic construct
MSPVQSLFLLLLWILGTKGDVVLTQTPSILSVTVGQSVSISCRSSQSLLDSDGNTYLYWFLQRPGQSPQRLIYLVSNLGSGAPNRFSGSGSGTDFTLKISGVEAEDLGVYYCMQATHAPWTFGGGTKLELK

SEQ ID NO: 9 - protein, 30 aa, synthetic construct
EVQLVESGGGLVQPGKSLKLSCSASGFTFS

SEQ ID NO: 10 - protein, 14 aa, synthetic construct
WIRQAPGKGLDWVA

SEQ ID NO: 11 - protein, 32 aa, synthetic construct
RFTISRDNAKSTLYLQLNSLKSEDTAIYYCAS

SEQ ID NO: 12 - protein, 11 aa, synthetic construct
WGQGVMVTVSS

SEQ ID NO: 13 - protein, 23 aa, synthetic construct
DVVLTQTPSILSVTVGQSVSISC

SEQ ID NO: 14 - protein, 15 aa, synthetic construct
WFLQRPGQSPQRLIY

SEQ ID NO: 15 - protein, 32 aa, synthetic construct
GAPNRFSGSGSGTDFTLKISGVEAEDLGVYYC

SEQ ID NO: 16 - protein, 10 aa, synthetic construct
FGGGTKLELK

SEQ ID NO: 17 - DNA, 405 bp, synthetic construct
  source 1..405: mol_type = other DNA
atgtacttcagcatcagcttgtttttccttgtgctcattttaaaaagtgtccagtgtgaggtacagctggtggagtctggaggaggcttagtgcagcctggaaagtccctgaaactctcctgttcagcctctggattcacattcagtaggtatggcatgcactggattcgccaagctccaggaaaggggctagattgggttgcatacattactcgtagcagcgatacagtctatgcagacgctgtgaagggccggttcaccatctccagagacaatgcaaagagcaccctgtacctgcaactcaacagtctgaagtctgaagacactgccatctattactgtgcaagtcactttgctacagtggaaagttactggggccaaggagtcatggtcacagtctcctca

SEQ ID NO: 18 - DNA, 393 bp, synthetic construct
  source 1..393: mol_type = other DNA
atgagtcctgtccagtccctgtttttattattgctttggattctgggaaccaaaggtgatgttgtgctgacccagactccatccatattgtctgttaccgttggacaatcggtctccatctcttgcaggtcaagtcagagtctcttagatagtgatggaaacacctatttatattggttcctacagaggccaggccagtctccacagcgtctaatttatttggtatccaacctgggatctggggcccccaacaggttcagtggcagtgggtcaggaacagatttcacactcaaaatcagtggagtggaggctgaggatttgggagtttattactgcatgcaagctacccatgctccgtggacgttcggtggaggtaccaagctggaattgaaa